European Patent Specification EP 3 083 682 B1, published April 17, 2024. Title: DUAL SPECIFIC ANTIBODIES. Applicant: Genentech, Inc. F. Hoffmann-La Roche AG. The sequence listing filed with the application follows.

SEQUENCE LISTING (34 sequences)

SEQ ID NO: 1 - protein, 107 aa, Artificial Sequence
  Synthetic Construct
DIQMTQSPSSLSASVGDRVTITCKASQSVINDAAWYQQKPGKAPKLLIYYTSHRYTGVPSRFSGSGSGTDFTLTISSLQEDFATYYCQQDYTSPWTFGQGTKVEIKR

SEQ ID NO: 2 - protein, 118 aa, Artificial Sequence
  Synthetic Construct
EVQLVQSGAEVKKPGASVKVSCKASGYTFTDYSMHWVRQAPGQGLEWIVWINTETGEPTYADDFKGRVTITRDTSTSTAYLELSSLRSEDTAVYYCARGGIFYGMDYWGQGTLVTVSS

SEQ ID NO: 3 - protein, 118 aa, Artificial Sequence
  Synthetic Construct
EVQLVQSGAEVKKPGASVKVSCKASGYTFTDYDIHWVRQAPGQGLEWIVWINTETGEPTYADDFKGRVTITRDTSTSTAYLELSSLRSEDTAVYYCAREILFYGMDYWGQGTLVTVSS

SEQ ID NO: 4 - protein, 119 aa, Artificial Sequence
  Synthetic Construct
EVQLVQSGAEVKKPGASVKVSCKASGYTFTDYFIHWVRQAPGQGLEWIAGIVYDATGFTTYADDFKGRVTITRDTSTSTAYLELSSLRSEDTAVYYCARGGIFYGMDYWGQGTLVTVSS

SEQ ID NO: 5 - protein, 108 aa, Artificial Sequence
  Synthetic Construct
DIQMTQSPSSLSASVGDRVTITCKASQSVINDAAWYQQKPGKAPKLLIYYTSHRYTGVPSRFSGSGSGTDFTLTISSLQEDFATYYCQQDYTPFPLTFGQGTKVEIKR

SEQ ID NO: 6 - protein, 118 aa, Artificial Sequence
  Synthetic Construct
EVQLVQSGAEVKKPGASVKVSCKASGYTFTDYLMHWVRQAPGQGLEWIAVIVSITGRTYYADDFKGRVTITRDTSTSTAYLELSSLRSEDTAVYYCARGGIFYGMDYWGQGTLVTVSS

SEQ ID NO: 7 - protein, 117 aa, Artificial Sequence
  Synthetic Construct
EVQLVQSGAEVKKPGASVKVSCKASGYTFTDYSMHWVRQAPGQGLEWIGVIFQSGATYYADDFKGRVTITRDTSTSTAYLELSSLRSEDTAVYYCARGGIFYGMDYWGQGTLVTVSS

SEQ ID NO: 8 - protein, 117 aa, Artificial Sequence
  Synthetic Construct
EVQLVQSGAEVKKPGASVKVSCKASGYTFTDYSMHWVRQAPGQGLEWIGIIFYTGHTYYADDFKGRVTITRDTSTSTAYLELSSLRSEDTAVYYCARGGIFYGMDYWGQGTLVTVSS

SEQ ID NO: 9 - protein, 11 aa, Artificial Sequence
  Synthetic Construct
KASQSVINDAA

SEQ ID NO: 10 - protein, 7 aa, Artificial Sequence
  Synthetic Construct
YTSHRYT

SEQ ID NO: 11 - protein, 10 aa, Artificial Sequence
  Synthetic Construct
QQDYTSPWTF

SEQ ID NO: 12 - protein, 11 aa, Artificial Sequence
  Synthetic Construct
QQDYTPFPLTF

SEQ ID NO: 13 - protein, 5 aa, Artificial Sequence
  Synthetic Construct
DYSMH

SEQ ID NO: 14 - protein, 5 aa, Artificial Sequence
  Synthetic Construct
DYDIH

SEQ ID NO: 15 - protein, 5 aa, Artificial Sequence
  Synthetic Construct
DYFIH

SEQ ID NO: 16 - protein, 5 aa, Artificial Sequence
  Synthetic Construct
DYLMH

SEQ ID NO: 17 - protein, 17 aa, Artificial Sequence
  Synthetic Construct
VWINTETGEPTYADDFK

SEQ ID NO: 18 - protein, 18 aa, Artificial Sequence
  Synthetic Construct
AGIVYDATGFTTYADDFK

SEQ ID NO: 19 - protein, 17 aa, Artificial Sequence
  Synthetic Construct
AVIVSITGRTYYADDFK

SEQ ID NO: 20 - protein, 9 aa, Artificial Sequence
  Synthetic Construct
GGIFYGMDY

SEQ ID NO: 21 - protein, 9 aa, Artificial Sequence
  Synthetic Construct
EILFYGMDY

SEQ ID NO: 22 - protein, 16 aa, Artificial Sequence
  Synthetic Construct
GVIFQSGATYYADDFK

SEQ ID NO: 23 - protein, 16 aa, Artificial Sequence
  Synthetic Construct
GIIFYTGHTYYADDFK

SEQ ID NO: 24 - protein, 10 aa, Artificial Sequence
  Synthetic Construct
  MISC_FEATURE (5)..(5): Xaa is Thr, Ile, Lys, or Leu
  MISC_FEATURE (6)..(6): Xaa is Ser or His
QQDYXXPWTF

SEQ ID NO: 25 - protein, 18 aa, Artificial Sequence
  Synthetic Construct
  MISC_FEATURE (1)..(1): Xaa is Ala or Gly
  MISC_FEATURE (12)..(12): Xaa is Thr, Ile, Val, or Ala
  MISC_FEATURE (15)..(15): Xaa is Asp, Val, or Glu
  MISC_FEATURE (16)..(16): Xaa is Asp, Glu, Asn, Ser, Ile, Leu, Thr, Ala, or Phe
XGIVYDATGFTXYAXXFK

SEQ ID NO: 26 - protein, 14 aa, Artificial Sequence
  Synthetic Construct
  MISC_FEATURE (3)..(3): Xaa is Val or Phe
  MISC_FEATURE (7)..(7): Xaa is Arg or Ile
  MISC_FEATURE (9)..(9): Xaa is Thr, Phe, Met, or Pro
  MISC_FEATURE (14)..(14): Xaa is Ala or Val.
GRXTITXDXSTSTX

SEQ ID NO: 27 - protein, 10 aa, Artificial Sequence
  Synthetic Construct
QQDYTHPWTF

SEQ ID NO: 28 - protein, 18 aa, Artificial Sequence
  Synthetic Construct
GGIVYDATGFTTYAEEFK

SEQ ID NO: 29 - protein, 107 aa, Artificial Sequence
  Synthetic Construct
DIQMTQSPSSLSASVGDRVTITCKASQSVINDAAWYQQKPGKAPKLLIYYTSHRYTGVPSRFSGSGSGTDFTLTISSLQEDFATYYCQQDYTHPWTFGQGTKVEIKR

SEQ ID NO: 30 - protein, 119 aa, Artificial Sequence
  Synthetic Construct
EVQLVQSGAEVKKPGASVKVSCKASGYTFTDYFIHWVRQAPGQGLEWIGGIVYDATGFTTYAEEFKGRVTITRDTSTSTAYLELSSLRSEDTAVYYCARGGIFYGMDYWGQGTLVTVSS

SEQ ID NO: 31 - protein, 10 aa, Artificial Sequence
  Synthetic Construct
QQDYKHPWTF

SEQ ID NO: 32 - protein, 18 aa, Artificial Sequence
  Synthetic Construct
AGIVYDATGFTVYADDFK

SEQ ID NO: 33 - protein, 107 aa, Artificial Sequence
  Synthetic Construct
DIQMTQSPSSLSASVGDRVTITCKASQSVINDAAWYQQKPGKAPKLLIYYTSHRYTGVPSRFSGSGSGTDFTLTISSLQEDFATYYCQQDYKHPWTFGQGTKVEIKR

SEQ ID NO: 34 - protein, 119 aa, Artificial Sequence
  Synthetic Construct
EVQLVQSGAEVKKPGASVKVSCKASGYTFTDYFIHWVRQAPGQGLEWIAGIVYDATGFTVYADDFKGRVTITRDTSTSTAYLELSSLRSEDTAVYYCARGGIFYGMDYWGQGTLVTVSS